European Patent Application EP 4 368 203 A1, published May 15, 2024. Title: 一种抗VEGF抗体体内表达系统的构建和应用. Applicant: 武汉纽福斯生物科技有限公司. Application CN. The sequence listing filed with the application follows.

SEQUENCE LISTING (35 sequences)

SEQ ID NO: 1 - DNA, 583 bp, synthetic construct
  source 1..583: mol_type = other DNA
cgttacataacttacggtaaatggcccgcctggctgaccgcccaacgacccccgcccattgacgtcaataatgacgtatgttcccatagtaacgccaatagggactttccattgacgtcaatgggtggagtatttacggtaaactgcccacttggcagtacatcaagtgtatcatatgccaagtacgccccctattgacgtcaatgacggtaaatggcccgcctggcattatgcccagtacatgaccttatgggactttcctacttggcagtacatctacgtattagtcatcgctattaccatggtcgaggtgagccccacgttctgcttcactctccccatctcccccccctccccacccccaattttgtatttatttattttttaattattttgtgcagcgatgggggcggggggggggggggggcgcgcgccaggcggggcggggcggggcgaggggcggggcggggcgaggcggagaggtgcggcggcagccaatcagagcggcgcgctccgaaagtttccttttatggcgaggcggcggcggcggcggccctataaaaagcgaagcgcgcggcgggcg

SEQ ID NO: 2 - DNA, 988 bp, synthetic construct
  source 1..988: mol_type = other DNA
cgcgttactcccacaggtgagcgggcgggacggcccttctcctccgggctgtaattagcgcttggtttaatgacggcttgtttcttttctgtggctgcgtgaaagccttgaggggctccgggagggccctttgtgcggggggagcggctcggggggtgcgtgcgtgtgtgtgtgcgtggggagcgccgcgtgcggctccgcgctgcccggcggctgtgagcgctgcgggcgcggcgcggggctttgtgcgctccgcagtgtgcgcgaggggagcgcggccgggggcggtgccccgcggtgcggggggggctgcgaggggaacaaaggctgcgtgcggggtgtgtgcgtgggggggtgagcagggggtgtgggcgcgtcggtcgggctgcaaccccccctgcacccccctccccgagttgctgagcacggcccggcttcgggtgcggggctccgtacggggcgtggcgcggggctcgccgtgccgggcggggggtggcggcaggtgggggtgccgggcggggcggggccgcctcgggccggggagggctcgggggaggggcgcggcggcccccggagcgccggcggctgtcgaggcgcggcgagccgcagccattgccttttatggtaatcgtgcgagagggcgcagggacttcctttgtcccaaatctgtgcggagccgaaatctgggaggcgccgccgcaccccctctagcgggcgcggggcgaagcggtgcggcgccggcaggaaggaaatgggcggggagggccttcgtgcgtcgccgcgccgccgtccccttctccctctccagcctcggggctgtccgcggggggacggctgccttcgggggggacggggcagggcggggttcggcttctggcgtgtgaccggcggctctagagcctctgctaaccatgttcatgccttcttctttttcctacagctcctgggcaacgtgctggttattgtgctgtctcatcattttggcaaa

SEQ ID NO: 3 - DNA, 1099 bp, synthetic construct
  source 1..1099: mol_type = other DNA
cgcgttactcccacaggtgagcgggcgggacggcccttctcctccgggctgtaattagcgcttggtttaatgacggcttgtttcttttctgtggctgcgtgaaagccttgaggggctccgggagggccctttgtgcggggggagcggctcggggggtgcgtgcgtgtgtgtgtgcgtggggagcgccgcgtgcggctccgcgctgcccggcggctgtgagcgctgcgggcgcggcgcggggctttgtgcgctccgcagtgtgcgcgaggggagcgcggccgggggcggtgccccgcggtgcggggggggctgcgaggggaacaaaggctgcgtgcggggtgtgtgcgtgggggggtgagcagggggtgtgggcgcgtcggtcgggctgcaaccccccctgcacccccctccccgagttgctgagcacggcccggcttcgggtgcggggctccgtacggggcgtggcgcggggctcgccgtgccgggcggggggtggcggcaggtgggggtgccgggcggggcggggccgcctcgggccggggagggctcgggggaggggcgcggcggcccccggagcgccggcggctgtcgaggcgcggcgagccgcagccattgccttttatggtaatcgtgcgagagggcgcagggacttcctttgtcccaaatctgtgcggagccgaaatctgggaggcgccgccgcaccccctctagcgggcgcggggcgaagcggtgcggcgccggcaggaaggaaatgggcggggagggccttcgtgcgtcgccgcgccgccgtccccttctccctctccagcctcggggctgtccgcggggggacggctgccttcgggggggacggggcagggcggggttcggcttctggcgtgtgaccggcggctctagagtaagtatcaaggttacaagacaggtttaaggagaccaatagaaactgggcttgtcgagacagagaagactcttgcgtttctgataggcacctattggtcttactgacatccactttgcctttctctccacaggtgtccactcccagttcaattacagctcttaaggctagagtacttaatacgactcactataggctagc

SEQ ID NO: 4 - DNA, 642 bp, synthetic construct
  source 1..642: mol_type = other DNA
gacatccagctgacccagtccccgagctccctgtccgcctctgtgggcgatagggtcaccatcacctgcagtgccagtcaagacatcagcaactatctgaactggtatcaacagaagccaggaaaggctccgaaggtactgatttactttaccagtagtctccatagtggagtcccttctcgcttctctggatccggttctgggacggatttcactctgaccatcagcagtctacagccagaagacttcgcaacttattactgtcaacagtacagtacggttccatggacatttggacagggcaccaaggtggagatcaaacgaactgtggctgcaccatctgtcttcatcttcccgccatctgatgagcagttgaaatctggaactgcttctgttgtgtgcctgctgaataacttctatcccagagaggccaaagtacagtggaaggtggataacgccctccaatcgggtaactcccaggagagtgtcacagagcaggacagcaaggacagcacctacagcctcagcagcaccctgacgctgagcaaagcagactacgagaaacacaaagtctacgcctgcgaagtcacccatcagggcctaagctcgcccgtcacaaagagcttcaacaggggagagtgt

SEQ ID NO: 5 - DNA, 693 bp, synthetic construct
  source 1..693: mol_type = other DNA
gaagtgcagctggtggagtctgggggaggcttggtacagcctggcgggtccctgagactctcctgtgcagcctctggatacgactttactcattatggcatgaactgggtccggcaagctccagggaagggcctggaatgggtcggatggattaatacctatacgggagaacctacttatgcggccgatttcaagcgccgattcaccttctccttagacacctccaagagcaccgcgtatttgcaaatgaacagtctgagagctgaggacacggccgtgtattactgtgcaaaatatccatattattatgggacatcgcactggtattttgacgtctggggccagggaaccctggtcaccgtctcctcagcctccaccaagggccctagcgtcttccccctggcaccctctagcaagagcacctccggaggcacagcggccctgggctgcctggtcaaggactacttccccgaaccggtgacggtgtcatggaactcaggcgccctgaccagcggcgtgcacaccttcccggctgtcctacagtcctcaggactctactccctcagcagcgtggtgaccgtgccctccagcagcttgggcacccagacctacatctgcaacgtgaatcacaagcccagcaacaccaaggtggacaagaaagttgagcccaagagttgtgacaaaactcacctt

SEQ ID NO: 6 - DNA, 708 bp, synthetic construct
  source 1..708: mol_type = other DNA
gaagtgcagctggtggagtctgggggaggcttggtacagcctggggggtccctgagactctcctgtgcagcctctggatacgactttactcattatggcatgaactgggtccggcaagctccagggaagggcctggaatgggtcggatggattaatacctatacgggagaacctacttatgcggccgatttcaagcgccgattcaccttctccttagacacctccaagagcaccgcgtatttgcaaatgaacagtctgagagctgaggacacggccgtgtattactgtgcaaaatatccatattattatgggacatcgcactggtattttgacgtctggggccagggaaccctggtcaccgtctcctcagcctccaccaagggccctagcgtcttccccctggcaccctctagcaagagcacctccggaggcacagcggccctgggctgcctggtcaaggactacttccccgaaccggtgacggtgtcatggaactcaggcgccctgaccagcggcgtgcacaccttcccggctgtcctacagtcctcaggactctactccctcagcagcgtggtgaccgtgccctccagcagcttgggcacccagacctacatctgcaacgtgaatcacaagcccagcaacaccaaggtggacaagaaagttgagcccaagagttgtgacaaaactcacctttgcccaccgtgccca

SEQ ID NO: 7 - DNA, 477 bp, Human
  source 1..477: mol_type = other DNA
gggtggcatccctgtgacccctccccagtgcctctcctggccctggaagttgccactccagtgcccaccagccttgtcctaataaaattaagttgcatcattttgtctgactaggtgtccttctataatattatggggtggaggggggtggtatggagcaaggggcaagttgggaagacaacctgtagggcctgcggggtctattgggaaccaagctggagtgcagtggcacaatcttggctcactgcaatctccgcctcctgggttcaagcgattctcctgcctcagcctcccgagttgttgggattccaggcatgcatgaccaggctcagctaatttttgtttttttggtagagacggggtttcaccatattggccaggctggtctccaactcctaatctcaggtgatctacccaccttggcctcccaaattgctgggattacaggcgtgaaccactgctcccttccctgtcctt

SEQ ID NO: 8 - protein, 20 aa, synthetic construct
MYRMQLLSCIALSLALVTNS

SEQ ID NO: 9 - protein, 20 aa, synthetic construct
MYRMQLLLLIALSLALVTNS

SEQ ID NO: 10 - protein, 26 aa, synthetic construct
MVSYWDTGVLLCARCSAVCFSQDLVP

SEQ ID NO: 11 - protein, 24 aa, synthetic construct
MSRKIEGFLLLLLFGYEATLGLSS

SEQ ID NO: 12 - protein, 26 aa, synthetic construct
MNFLLSWVHWSLALLLYLHHAKWSQA

SEQ ID NO: 13 - protein, 18 aa, synthetic construct
MKWVTFISLLFLFSSAYS

SEQ ID NO: 14 - protein, 28 aa, synthetic construct
RARRAPVKQTLNFDLLKLAGDVESNPGP

SEQ ID NO: 15 - protein, 35 aa, synthetic construct
CPPCPAPRKRRAPVKQTLNFDLLKLAGDVESNPGP

SEQ ID NO: 16 - protein, 214 aa, synthetic construct
DIQLTQSPSSLSASVGDRVTITCSASQDISNYLNWYQQKPGKAPKVLIYFTSSLHSGVPSRFSGSGSGTDFTLTISSLQPEDFATYYCQQYSTVPWTFGQGTKVEIKRTVAAPSVFIFPPSDEQLKSGTASVVCLLNNFYPREAKVQWKVDNALQSGNSQESVTEQDSKDSTYSLSSTLTLSKADYEKHKVYACEVTHQGLSSPVTKSFNRGEC

SEQ ID NO: 17 - protein, 231 aa, synthetic construct
EVQLVESGGGLVQPGGSLRLSCAASGYDFTHYGMNWVRQAPGKGLEWVGWINTYTGEPTYAADFKRRFTFSLDTSKSTAYLQMNSLRAEDTAVYYCAKYPYYYGTSHWYFDVWGQGTLVTVSSASTKGPSVFPLAPSSKSTSGGTAALGCLVKDYFPEPVTVSWNSGALTSGVHTFPAVLQSSGLYSLSSVVTVPSSSLGTQTYICNVNHKPSNTKVDKKVEPKSCDKTHL

SEQ ID NO: 18 - protein, 236 aa, synthetic construct
EVQLVESGGGLVQPGGSLRLSCAASGYDFTHYGMNWVRQAPGKGLEWVGWINTYTGEPTYAADFKRRFTFSLDTSKSTAYLQMNSLRAEDTAVYYCAKYPYYYGTSHWYFDVWGQGTLVTVSSASTKGPSVFPLAPSSKSTSGGTAALGCLVKDYFPEPVTVSWNSGALTSGVHTFPAVLQSSGLYSLSSVVTVPSSSLGTQTYICNVNHKPSNTKVDKKVEPKSCDKTHLCPPCP

SEQ ID NO: 19 - DNA, 642 bp, synthetic construct
  source 1..642: mol_type = other DNA
gatatccagctcactcaatccccttctagcctgagtgcctcagtgggggaccgcgtcacaatcacctgctccgcttcccaggacatcagtaactacctcaattggtaccagcagaagccaggcaaggccccaaaggttctgatctactttacatcatccctccactcaggggtcccgtctcggttttccggaagcggctccggaaccgacttcacgcttactatctccagtctccagccagaagatttcgcaacatactactgccagcagtatagcacagttccatggactttcggccagggcaccaaagtggaaataaagagaaccgtggccgccccatctgtgttcatattccccccaagtgacgagcaactgaagagcgggacggcgtccgttgtgtgcctcttgaataatttctatcctagagaagccaaggttcaatggaaggtggataacgccctgcagtcaggcaacagccaggagtccgtgacagagcaagacagtaaggattccacatatagcctttcttccaccctgacacttagtaaggcagactacgaaaaacacaaagtatatgcctgcgaagtgacacaccaagggctgtctagccccgttactaagtcctttaatagaggagagtgc

SEQ ID NO: 20 - DNA, 642 bp, synthetic construct
  source 1..642: mol_type = other DNA
gatatacagttgacacagagtcctagctctctttccgcttcagtcggcgaccgggtcaccataacctgtagtgcatcccaggacataagcaattatcttaattggtaccagcaaaaaccaggaaaagcgcctaaagttctgatctactttacgagttccctgcattctggcgttcccagtcgattttcaggttcaggctccgggacagactttacacttactattagcagcctccagccggaggattttgccacctattattgtcaacaatattcaactgttccatggacctttgggcaaggcactaaagtggaaattaagcggactgtagctgcgcctagcgtatttatatttccgccgtccgatgaacaactcaagtcaggcacggcgagcgtggtttgccttctcaacaatttctatccaagggaggccaaggtgcagtggaaagttgacaatgccttgcaatctggcaacagtcaagaaagcgttactgaacaggactccaaggatagtacgtacagcctcagctcaacactcaccctttccaaggccgattacgagaaacataaggtctatgcgtgtgaagttactcaccagggcctgagtagccccgtaaccaagagcttcaatcgcggggaatgt

SEQ ID NO: 21 - DNA, 642 bp, synthetic construct
  source 1..642: mol_type = other DNA
gacattcagctgacacagagccctagcagcctgtctgcctctgtgggagacagagtgaccatcacctgtagcgccagccaggacatcagcaactacctgaactggtatcagcagaagcccggcaaggcccctaaggtgctgatctactttaccagcagcctgcactccggcgtgcccagcagattttctggctctggcagcggcaccgacttcaccctgaccatatctagcctgcagcctgaggacttcgccacctactactgccagcagtacagcaccgtgccttggacatttggccagggcacaaaggtggaaatcaagcggacagtggccgctcctagcgtgttcatctttccacctagcgacgagcagctgaagtctggcacagcctctgtcgtgtgcctgctgaacaacttctaccccagagaagccaaggtgcagtggaaagtggacaacgccctgcagagcggcaacagccaagagtctgtgaccgagcaggacagcaaggactccacctatagcctgagcagcaccctgacactgagcaaggccgactacgagaagcacaaagtgtacgcctgcgaagtgacccaccagggcctttctagccctgtgaccaagagcttcaaccggggcgagtgt

SEQ ID NO: 22 - DNA, 642 bp, synthetic construct
  source 1..642: mol_type = other DNA
gatatccagctgacccagtccccaagtagcctgagcgcctccgtcggagatagagtgacaatcacctgcagcgccagccaggacatcagcaactacctgaactggtatcagcaaaaacctggaaaggcccctaaggttctgatctactttacaagcagcctgcacagcggagtaccctccagattcagcggatctggctccggcactgatttcaccctgaccattagctcactgcagcctgaggatttcgccacatactattgtcagcagtactccacagtcccttggaccttcggccagggcaccaaagtggagatcaagaggaccgtggctgctcccagcgtgttcatcttcccccccagcgacgagcagctgaaaagcggtaccgcctctgtggtgtgcctgctgaacaacttctacccgcgggaagctaaggtgcagtggaaggtggacaacgccctgcagagcggcaatagccaggagagcgtgaccgagcaggattctaaagacagcacctactctctgtcttctaccctgaccctgtcaaaggccgactacgagaagcacaaggtgtacgcctgcgaggtgacacatcagggcctgagcagccctgtgacaaagagcttcaacagaggcgagtgt

SEQ ID NO: 23 - DNA, 693 bp, synthetic construct
  source 1..693: mol_type = other DNA
gaggtgcaattggtcgagtccggggggggcctcgtgcaaccaggaggttccctcaggctgagctgtgccgcaagcggatacgatttcacccactacgggatgaactgggtgagacaggcccccgggaaaggcctcgagtgggtcggatggataaacacatacaccggagagcccacctacgcagccgactttaaaagaagatttaccttctccctggataccagcaagtccacagcctaccttcagatgaactccctgagagcagaggatacggcggtctattactgcgccaaatacccttattattatggaaccagtcattggtacttcgatgtgtggggtcagggcacactcgtgacggtgtcaagtgcttccacgaaagggccatctgtgtttcctctcgcccccagctccaaatctactagtggcggcaccgccgccctcggatgtctcgtcaaagactacttccccgaaccagttaccgttagctggaacagcggcgccttgaccagtggggtgcatacatttccagccgtgttgcagagcagcggcctgtattccctgagcagtgtggtaacagtcccatcctcttctctgggaacccaaacttacatatgtaatgtgaaccacaaaccatcaaataccaaagtcgataaaaaagtagaacctaagagctgcgataaaacacacctc

SEQ ID NO: 24 - DNA, 693 bp, synthetic construct
  source 1..693: mol_type = other DNA
gaagttcagcttgtcgagtctggaggaggacttgtgcagcccggcggatccctgcgactctcatgcgctgctagtgggtatgattttactcactatggaatgaattgggtccgacaagctcccggaaaaggcttggaatgggtcggatggattaacacatacactggagagccgacgtatgctgcagattttaaaaggcgatttaccttcagcctggacactagcaagtcaaccgcatacctccagatgaattccctcagggctgaagacactgcagtgtattattgtgcaaaatacccttattattacggtacctcccattggtatttcgatgtgtgggggcaaggtacgctggttactgtgtcaagtgcgtcaacaaagggaccatctgtattccccctcgcaccaagctcaaagagtacatccggagggactgcagccttgggctgtttggttaaggactacttcccagagcctgttaccgtctcctggaactcaggtgcccttacgtcaggcgttcatacatttcctgccgtgctgcagtcttccgggctttacagtttgagttctgtggtaacagtaccgagtagcagcctcggtactcagacttacatctgcaatgttaaccataaaccttccaacacaaaagtggacaagaaggtagagcccaagagttgcgataaaacgcacttg

SEQ ID NO: 25 - DNA, 693 bp, synthetic construct
  source 1..693: mol_type = other DNA
gaggtgcagctggttgaatctggcggaggactggttcagcctggcggatctctgagactgtcttgtgccgccagcggctacgactttacccactacggcatgaactgggtccgacaggcccctggcaaaggccttgaatgggtcggatggatcaacacctacaccggcgagccaacatacgccgccgacttcaagcggagattcacctttagcctggacaccagcaagagcaccgcctacctgcagatgaacagcctgagagccgaggacaccgccgtgtactactgcgccaagtatccctactactacggcaccagccactggtacttcgacgtgtggggacagggcacactggtcacagtgtctagcgcctctacaaagggccccagcgttttcccactggctcctagcagcaagtctaccagcggaggaacagccgctctgggctgtctggtcaaggactactttcccgagcctgtgaccgtgtcctggaattctggcgctctgacaagcggcgtgcacacctttccagctgtgctgcaaagcagcggcctgtactctctgagcagcgtcgtgacagtgccaagcagctctctgggcacccagacctacatctgcaatgtgaaccacaagcctagcaacaccaaggtggacaagaaggtggaacccaagagctgcgacaagacccacctg

SEQ ID NO: 26 - DNA, 693 bp, synthetic construct
  source 1..693: mol_type = other DNA
gaagttcaactggtggaatctggaggcggcctggtgcagcctggcggaagccttagactgtcgtgcgccgccagtggctacgacttcacccactacggcatgaattgggtgcggcaggcccctggcaagggcctggaatgggtgggctggatcaacacctatacaggcgagcctacatatgccgctgatttcaagcggagattcaccttcagcctggacaccagcaagagcacagcctacctgcagatgaacagcctgcgcgccgaggacacagccgtgtactactgcgccaagtacccctactactacggcaccagccactggtacttcgacgtgtggggccaaggaacgctggtgaccgtgtcgagcgccagcacaaagggccctagcgtgttccccctggcccctagcagcaaaagcaccagcggcggcaccgccgccctgggctgcctggtgaaggactactttcctgagcctgtgacagtcagctggaactcgggagccctgacaagcggcgtgcacacctttcctgctgtgctgcagagctctggactgtactctctgagcagcgtcgtgaccgtgccaagttcttctctcggcacccagacctacatctgcaacgtgaaccacaagccttccaacaccaaggtggataagaaagtggaacccaagagctgcgacaagacccacctg

SEQ ID NO: 27 - DNA, 542 bp, Woodchuck hepatitis virus
  source 1..542: mol_type = genomic DNA
aatcaacctctggattacaaaatttgtgaaagattgactggtattcttaactatgttgctccttttacgctatgtggatacgctgctttaatgcctttgtatcatgctattgcttcccgtatggctttcattttctcctccttgtataaatcctggttgctgtctctttatgaggagttgtggcccgttgtcaggcaacgtggcgtggtgtgcactgtgtttgctgacgcaacccccactggttggggcattgccaccacctgtcagctcctttccgggactttcgctttccccctccctattgccacggcggaactcatcgccgcctgccttgcccgctgctggacaggggctcggctgttgggcactgacaattccgtggtgttgtcggggaagctgtggtcctttccagggctgctcgcctgtgttgccacctggattctgcgcgggacgtccttctgctacgtcccttcggccctcaatccagcggaccttccttcccgcggcctgctgccggctctgcggcctcttccgcgtcttcg

SEQ ID NO: 28 - protein, 11 aa, synthetic construct
SASQDISNYLN

SEQ ID NO: 29 - protein, 7 aa, synthetic construct
FTSSLHS

SEQ ID NO: 30 - protein, 9 aa, synthetic construct
QQYSTVPWT

SEQ ID NO: 31 - protein, 10 aa, synthetic construct
GYDFTHYGMN

SEQ ID NO: 32 - protein, 17 aa, synthetic construct
WINTYTGEPTYAADFKR

SEQ ID NO: 33 - protein, 14 aa, synthetic construct
YPYYYGTSHWYFDV

SEQ ID NO: 34 - protein, 19 aa, synthetic construct
MEFGLSWVFLVAILKGVQC

SEQ ID NO: 35 - protein, 25 aa, synthetic construct
MKKNIAFLLASMFVFSIATNAYAEV